European Patent Application EP 4 606 821 A1, published August 27, 2025. Title: FcεRI BINDING PROTEIN. Applicant: LONGBIO PHARMA (SUZHOU) CO., LTD. The sequence listing filed with the application follows.

SEQUENCE LISTING (42 sequences)

SEQ ID NO: 1 - protein, 10 aa, synthetic construct
  REGION 1..10: note = IgG Fc CH2 BC-LOOP-1
DVSHEDPEVK

SEQ ID NO: 2 - protein, 10 aa, synthetic construct
  REGION 1..10: note = IgG Fc CH2 BC-LOOP-2
DVSHEDPEVQ

SEQ ID NO: 3 - protein, 8 aa, synthetic construct
  REGION 1..8: note = IgG Fc CH2 DE-TURN-1
EQYNSTYR

SEQ ID NO: 4 - protein, 8 aa, synthetic construct
  REGION 1..8: note = IgG Fc CH2 DE-TURN-2
EQFNSTYR

SEQ ID NO: 5 - protein, 11 aa, synthetic construct
  REGION 1..11: note = IgG Fc CH2 FG-LOOP-1
KVSNKALPAPI

SEQ ID NO: 6 - protein, 11 aa, synthetic construct
  REGION 1..11: note = IgG Fc CH2 FG-LOOP-2
KVSNKGLPAPI

SEQ ID NO: 7 - protein, 11 aa, synthetic construct
  REGION 1..11: note = IgG Fc CH2 FG-LOOP-3
KVSNKGLPSSI

SEQ ID NO: 8 - protein, 10 aa, synthetic construct
  REGION 1..10: note = IgE Fc CH3 BC-LOOP
DLAPSKGTVN

SEQ ID NO: 9 - protein, 8 aa, synthetic construct
  REGION 1..8: note = IgE Fc CH3 DE-TURN
KQRNGTLT

SEQ ID NO: 10 - protein, 11 aa, synthetic construct
  REGION 1..11: note = IgE Fc CH3 FG-LOOP
RVTHPHLPRAL

SEQ ID NO: 11 - protein, 109 aa, synthetic construct
  REGION 1..109: note = IgG Fc CH2 (after mutation)
DSNPRGVSVFLFPPKPKDTLMISRTPEVTCVVVDLAPSKGTVKFNWYVDGVEVHNAKTKPREKQRNGTLTVVSVLTVLHQDWLNGKEYKCKVTHPHLPRALEKTISKAK

SEQ ID NO: 12 - protein, 110 aa, synthetic construct
  REGION 1..110: note = IgE fragment 1
DFTPPTVKILQSSCDGGGHFPPTIQLLCLVSGYTPGTINITWLEDGQVMDVDLSTASTTQEGELASTQSELTLSQKHWLSDRTYTCQVTYQGHTFEDSTKKCADSNPRGV

SEQ ID NO: 13 - protein, 113 aa, synthetic construct
  REGION 1..113: note = IgE fragment 2
CSRDFTPPTVKILQSSCDGGGHFPPTIQLLCLVSGYTPGTINITWLEDGQVMDVDLSTASTTQEGELASTQSELTLSQKHWLSDRTYTCQVTYQGHTFEDSTKKCADSNPRGV

SEQ ID NO: 14 - protein, 9 aa, synthetic construct
  REGION 1..9: note = IgE fragment 3
CADSNPRGV

SEQ ID NO: 15 - protein, 12 aa, synthetic construct
  REGION 1..12: note = IgE fragment 4
TKKCADSNPRGV

SEQ ID NO: 16 - protein, 322 aa, synthetic construct
  REGION 1..322: note = DB177
CSRDFTPPTVKILQSSCDGGGHFPPTIQLLCLVSGYTPGTINITWLEDGQVMDVDLSTASTTQEGELASTQSELTLSQKHWLSDRTYTCQVTYQGHTFEDSTKKCADSNPRGVSVFLFPPKPKDTLMISRTPEVTCVVVDLAPSKGTVKFNWYVDGVEVHNAKTKPREKQRNGTLTVVSVLTVLHQDWLNGKEYKCKVTHPHLPRALEKTISKAKGQPREPQVYTLPPSREEMTKNQVSLTCLVKGFYPSDIAVEWESNGQPENNYKTTPPVLDSDGSFFLYSKLTVDKSRWQQGNVFSCSVMHEALHNHYTQKSLSLSPGK

SEQ ID NO: 17 - protein, 319 aa, synthetic construct
  REGION 1..319: note = DB364
DFTPPTVKILQSSCDGGGHFPPTIQLLCLVSGYTPGTINITWLEDGQVMDVDLSTASTTQEGELASTQSELTLSQKHWLSDRTYTCQVTYQGHTFEDSTKKCADSNPRGVSVFLFPPKPKDTLMISRTPEVTCVVVDLAPSKGTVKFNWYVDGVEVHNAKTKPREKQRNGTLTVVSVLTVLHQDWLNGKEYKCKVTHPHLPRALEKTISKAKGQPREPQVYTLPPSREEMTKNQVSLTCLVKGFYPSDIAVEWESNGQPENNYKTTPPVLDSDGSFFLYSKLTVDKSRWQQGNVFSCSVMHEALHNHYTQKSLSLSPGK

SEQ ID NO: 18 - protein, 221 aa, synthetic construct
  REGION 1..221: note = DB365
TKKCADSNPRGVSVFLFPPKPKDTLMISRTPEVTCVVVDLAPSKGTVKFNWYVDGVEVHNAKTKPREKQRNGTLTVVSVLTVLHQDWLNGKEYKCKVTHPHLPRALEKTISKAKGQPREPQVYTLPPSREEMTKNQVSLTCLVKGFYPSDIAVEWESNGQPENNYKTTPPVLDSDGSFFLYSKLTVDKSRWQQGNVFSCSVMHEALHNHYTQKSLSLSPGK

SEQ ID NO: 19 - protein, 218 aa, synthetic construct
  REGION 1..218: note = DB366
CADSNPRGVSVFLFPPKPKDTLMISRTPEVTCVVVDLAPSKGTVKFNWYVDGVEVHNAKTKPREKQRNGTLTVVSVLTVLHQDWLNGKEYKCKVTHPHLPRALEKTISKAKGQPREPQVYTLPPSREEMTKNQVSLTCLVKGFYPSDIAVEWESNGQPENNYKTTPPVLDSDGSFFLYSKLTVDKSRWQQGNVFSCSVMHEALHNHYTQKSLSLSPGK

SEQ ID NO: 20 - protein, 543 aa, synthetic construct
  REGION 1..543: note = DB-871 heavy chain
EVQLVESGGGLVQPGGSLRLSCAASGFTFTDYTMDWVRQAPGKGLEWVADVNPNSGGSIYNQRFKGRFTLSVDRSKNTLYLQMNSLRAEDTAVYYCARNLGPSFYFDYWGQGTLVTVSSASTKGPSVFPLAPSSKSTSGGTAALGCLVKDYFPEPVTVSWNSGALTSGVHTFPAVLQSSGLYSLSSVVTVPSSSLGTQTYICNVNHKPSNTKVDKKVEPKSCSRDFTPPTVKILQSSCDGGGHFPPTIQLLCLVSGYTPGTINITWLEDGQVMDVDLSTASTTQEGELASTQSELTLSQKHWLSDRTYTCQVTYQGHTFEDSTKKCADSNPRGVSVFLFPPKPKDTLMISRTPEVTCVVVDLAPSKGTVKFNWYVDGVEVHNAKTKPREKQRNGTLTVVSVLTVLHQDWLNGKEYKCKVTHPHLPRALEKTISKAKGQPREPQVYTLPPSREEMTKNQVSLTCLVKGFYPSDIAVEWESNGQPENNYKTTPPVLDSDGSFFLYSKLTVDKSRWQQGNVFSCSVMHEALHNHYTQKSLSLSPGK

SEQ ID NO: 21 - protein, 449 aa, synthetic construct
  REGION 1..449: note = DB-872 heavy chain
EVQLVESGGGLVQPGGSLRLSCAASGFTFTDYTMDWVRQAPGKGLEWVADVNPNSGGSIYNQRFKGRFTLSVDRSKNTLYLQMNSLRAEDTAVYYCARNLGPSFYFDYWGQGTLVTVSSASTKGPSVFPLAPSSKSTSGGTAALGCLVKDYFPEPVTVSWNSGALTSGVHTFPAVLQSSGLYSLSSVVTVPSSSLGTQTYICNVNHKPSNTKVDKKVEPKSCDKTHTCPPCPADSNPRGVSVFLFPPKPKDTLMISRTPEVTCVVVDLAPSKGTVKFNWYVDGVEVHNAKTKPREKQRNGTLTVVSVLTVLHQDWLNGKEYKCKVTHPHLPRALEKTISKAKGQPREPQVYTLPPSREEMTKNQVSLTCLVKGFYPSDIAVEWESNGQPENNYKTTPPVLDSDGSFFLYSKLTVDKSRWQQGNVFSCSVMHEALHNHYTQKSLSLSPGK

SEQ ID NO: 22 - protein, 214 aa, synthetic construct
  REGION 1..214: note = DB-871/872 light chain
DIQMTQSPSSLSASVGDRVTITCKASQDVSIGVAWYQQKPGKAPKLLIYSASYRYTGVPSRFSGSGSGTDFTLTISSLQPEDFATYYCQQYYIYPYTFGQGTKVEIKRTVAAPSVFIFPPSDEQLKSGTASVVCLLNNFYPREAKVQWKVDNALQSGNSQESVTEQDSKDSTYSLSSTLTLSKADYEKHKVYACEVTHQGLSSPVTKSFNRGEC

SEQ ID NO: 23 - protein, 437 aa, synthetic construct
  REGION 1..437: note = FcRIa-mG2Ahis
MAPAMESPTLLCVALLFFAPDGVLAVPQKPKVSLNPPWNRIFKGENVTLTCNGNNFFEVSSTKWFHNGSLSEETNSSLNIVNAKFEDSGEYKCQHQQVNESEPVYLEVFSDWLLLQASAEVVMEGQPLFLRCHGWRNWDVYKVIYYKDGEALKYWYENHNISITNATVEDSGTYYCTGKVWQLDYESEPLNITVIKAPEPRGPTIKPCPPCKCPAPNLLGGPSVFIFPPKIKDVLMISLSPIVTCVVVDVSEDDPDVQISWFVNNVEVHTAQTQTHREDYNSTLRVVSALPIQHQDWMSGKEFKCKVNNKDLPAPIERTISKPKGSVRAPQVYVLPPPEEEMTKKQVTLTCMVTDFMPEDIYVEWTNNGKTELNYKNTEPVLDSDGSYFMYSKLRVEKKNWVERNSYSCSVVHEGLHNHHTTKSFSRTPGKHHHHHH

SEQ ID NO: 24 - protein, 110 aa, synthetic construct
  REGION 1..110: note = IgG Fc CH2 -1
APELLGGPSVFLFPPKPKDTLMISRTPEVTCVVVDVSHEDPEVKFNWYVDGVEVHNAKTKPREEQYNSTYRVVSVLTVLHQDWLNGKEYKCKVSNKALPAPIEKTISKAK

SEQ ID NO: 25 - protein, 109 aa, synthetic construct
  REGION 1..109: note = IgG Fc CH2 -2
APPVAGPSVFLFPPKPKDTLMISRTPEVTCVVVDVSHEDPEVQFNWYVDGVEVHNAKTKPREEQFNSTFRVVSVLTVVHQDWLNGKEYKCKVSNKGLPAPIEKTISKTK

SEQ ID NO: 26 - protein, 110 aa, synthetic construct
  REGION 1..110: note = IgG Fc CH2 -3
APELLGGPSVFLFPPKPKDTLMISRTPEVTCVVVDVSHEDPEVQFKWYVDGVEVHNAKTKPREEQYNSTFRVVSVLTVLHQDWLNGKEYKCKVSNKALPAPIEKTISKTK

SEQ ID NO: 27 - protein, 110 aa, synthetic construct
  REGION 1..110: note = IgG Fc CH2 -4
APEFLGGPSVFLFPPKPKDTLMISRTPEVTCVVVDVSQEDPEVQFNWYVDGVEVHNAKTKPREEQFNSTYRVVSVLTVLHQDWLNGKEYKCKVSNKGLPSSIEKTISKAK

SEQ ID NO: 28 - protein, 19 aa, synthetic construct
  REGION 1..19: note = Signal peptide
MGWSCIILFLVATATGVHS

SEQ ID NO: 29 - protein, 209 aa, synthetic construct
  REGION 1..209: note = IgG Fc(after mutation)
SVFLFPPKPKDTLMISRTPEVTCVVVDLAPSKGTVKFNWYVDGVEVHNAKTKPREKQRNGTLTVVSVLTVLHQDWLNGKEYKCKVTHPHLPRALEKTISKAKGQPREPQVYTLPPSREEMTKNQVSLTCLVKGFYPSDIAVEWESNGQPENNYKTTPPVLDSDGSFFLYSKLTVDKSRWQQGNVFSCSVMHEALHNHYTQKSLSLSPGK

SEQ ID NO: 30 - protein, 218 aa, synthetic construct
  REGION 1..218: note = DB-B63
CADSNPRGVSVFLFPPKPKDTLMISRTPEVTCVVVDLAPSKGTVNFNWYVDGVEVHNAKTKPREKQRNGTLTVVSVLTVLHQDWLNGKEYKCRVTHPHLPRALEKTISKAKGQPREPQVYTLPPSREEMTKNQVSLTCLVKGFYPSDIAVEWESNGQPENNYKTTPPVLDSDGSFFLYSKLTVDKSRWQQGNVFSCSVMHEALHNHYTQKSLSLSPGK

SEQ ID NO: 31 - protein, 219 aa, synthetic construct
  REGION 1..219: note = DB-B64
CPAPELLGGPSVFLFPPKPKDTLMISRTPEVTCVVVDLAPSKGTVKFNWYVDGVEVHNAKTKPREKQRNGTLTVVSVLTVLHQDWLNGKEYKCKVTHPHLPRALEKTISKAKGQPREPQVYTLPPSREEMTKNQVSLTCLVKGFYPSDIAVEWESNGQPENNYKTTPPVLDSDGSFFLYSKLTVDKSRWQQGNVFSCSVMHEALHNHYTQKSLSLSPGK

SEQ ID NO: 32 - protein, 539 aa, synthetic construct
  REGION 1..539: note = DB-B229 heavy chain
QVQLVQSGAEVKKPGASVKVSCKASGYTFTDYEMHWVRQAPGQGLEWMGALDPKTGDTAYSQKFKGRVTLTADKSTSTAYMELSSLTSEDTAVYYCTRFYSYTYWGQGTLVTVSSASTKGPSVFPLAPSSKSTSGGTAALGCLVKDYFPEPVTVSWNSGALTSGVHTFPAVLQSSGLYSLSSVVTVPSSSLGTQTYICNVNHKPSNTKVDKKVEPKSCSRDFTPPTVKILQSSCDGGGHFPPTIQLLCLVSGYTPGTINITWLEDGQVMDVDLSTASTTQEGELASTQSELTLSQKHWLSDRTYTCQVTYQGHTFEDSTKKCADSNPRGVSVFLFPPKPKDTLMISRTPEVTCVVVDLAPSKGTVKFNWYVDGVEVHNAKTKPREKQRNGTLTVVSVLTVLHQDWLNGKEYKCKVTHPHLPRALEKTISKAKGQPREPQVYTLPPSREEMTKNQVSLTCLVKGFYPSDIAVEWESNGQPENNYKTTPPVLDSDGSFFLYSKLTVDKSRWQQGNVFSCSVMHEALHNHYTQKSLSLSPGK

SEQ ID NO: 33 - protein, 445 aa, synthetic construct
  REGION 1..445: note = DB-B230 heavy chain
QVQLVQSGAEVKKPGASVKVSCKASGYTFTDYEMHWVRQAPGQGLEWMGALDPKTGDTAYSQKFKGRVTLTADKSTSTAYMELSSLTSEDTAVYYCTRFYSYTYWGQGTLVTVSSASTKGPSVFPLAPSSKSTSGGTAALGCLVKDYFPEPVTVSWNSGALTSGVHTFPAVLQSSGLYSLSSVVTVPSSSLGTQTYICNVNHKPSNTKVDKKVEPKSCDKTHTCPPCPADSNPRGVSVFLFPPKPKDTLMISRTPEVTCVVVDLAPSKGTVKFNWYVDGVEVHNAKTKPREKQRNGTLTVVSVLTVLHQDWLNGKEYKCKVTHPHLPRALEKTISKAKGQPREPQVYTLPPSREEMTKNQVSLTCLVKGFYPSDIAVEWESNGQPENNYKTTPPVLDSDGSFFLYSKLTVDKSRWQQGNVFSCSVMHEALHNHYTQKSLSLSPGK

SEQ ID NO: 34 - protein, 219 aa, synthetic construct
  REGION 1..219: note = DB-B229/DB-B230 light chain
DVVMTQSPLSLPVTPGEPASISCRSSQSLVHSNRNTYLHWYLQKPGQSPQLLIYKVSNRFSGVPDRFSGSGSGTDFTLKISRVEAEDVGVYYCSQNTHVPPTFGQGTKLEIKRTVAAPSVFIFPPSDEQLKSGTASVVCLLNNFYPREAKVQWKVDNALQSGNSQESVTEQDSKDSTYSLSSTLTLSKADYEKHKVYACEVTHQGLSSPVTKSFNRGEC

SEQ ID NO: 35 - protein, 545 aa, synthetic construct
  REGION 1..545: note = DB-B232 heavy chain
QVQLQQPGAELVKPGASVKMSCKASGYTFTSYNMHWVKQTPGRGLEWIGAIYPGNGDTSYNQKFKGKATLTADKSSSTAYMQLSSLTSEDSAVYYCARSTYYGGDWYFNVWGAGTTVTVSAASTKGPSVFPLAPSSKSTSGGTAALGCLVKDYFPEPVTVSWNSGALTSGVHTFPAVLQSSGLYSLSSVVTVPSSSLGTQTYICNVNHKPSNTKVDKKVEPKSCSRDFTPPTVKILQSSCDGGGHFPPTIQLLCLVSGYTPGTINITWLEDGQVMDVDLSTASTTQEGELASTQSELTLSQKHWLSDRTYTCQVTYQGHTFEDSTKKCADSNPRGVSVFLFPPKPKDTLMISRTPEVTCVVVDLAPSKGTVKFNWYVDGVEVHNAKTKPREKQRNGTLTVVSVLTVLHQDWLNGKEYKCKVTHPHLPRALEKTISKAKGQPREPQVYTLPPSREEMTKNQVSLTCLVKGFYPSDIAVEWESNGQPENNYKTTPPVLDSDGSFFLYSKLTVDKSRWQQGNVFSCSVMHEALHNHYTQKSLSLSPGK

SEQ ID NO: 36 - protein, 451 aa, synthetic construct
  REGION 1..451: note = DB-B233 heavy chain
QVQLQQPGAELVKPGASVKMSCKASGYTFTSYNMHWVKQTPGRGLEWIGAIYPGNGDTSYNQKFKGKATLTADKSSSTAYMQLSSLTSEDSAVYYCARSTYYGGDWYFNVWGAGTTVTVSAASTKGPSVFPLAPSSKSTSGGTAALGCLVKDYFPEPVTVSWNSGALTSGVHTFPAVLQSSGLYSLSSVVTVPSSSLGTQTYICNVNHKPSNTKVDKKVEPKSCDKTHTCPPCPADSNPRGVSVFLFPPKPKDTLMISRTPEVTCVVVDLAPSKGTVKFNWYVDGVEVHNAKTKPREKQRNGTLTVVSVLTVLHQDWLNGKEYKCKVTHPHLPRALEKTISKAKGQPREPQVYTLPPSREEMTKNQVSLTCLVKGFYPSDIAVEWESNGQPENNYKTTPPVLDSDGSFFLYSKLTVDKSRWQQGNVFSCSVMHEALHNHYTQKSLSLSPGK

SEQ ID NO: 37 - protein, 213 aa, synthetic construct
  REGION 1..213: note = DB-B232/DB-B233 light chain
QIVLSQSPAILSASPGEKVTMTCRASSSVSYIHWFQQKPGSSPKPWIYATSNLASGVPVRFSGSGSGTSYSLTISRVEAEDAATYYCQQWTSNPPTFGGGTKLEIKRTVAAPSVFIFPPSDEQLKSGTASVVCLLNNFYPREAKVQWKVDNALQSGNSQESVTEQDSKDSTYSLSSTLTLSKADYEKHKVYACEVTHQGLSSPVTKSFNRGEC

SEQ ID NO: 38 - protein, 209 aa, synthetic construct
  REGION 1..209: note = IgG Fc-2(after mutation)
SVFLFPPKPKDTLMISRTPEVTCVVVDLAPSKGTVNFNWYVDGVEVHNAKTKPREKQRNGTLTVVSVLTVLHQDWLNGKEYKCRVTHPHLPRALEKTISKAKGQPREPQVYTLPPSREEMTKNQVSLTCLVKGFYPSDIAVEWESNGQPENNYKTTPPVLDSDGSFFLYSKLTVDKSRWQQGNVFSCSVMHEALHNHYTQKSLSLSPGK

SEQ ID NO: 39 - protein, 8 aa, synthetic construct
  REGION 1..8: note = IgG Fc CH2 DE-TURN-3
EQFNSTFR

SEQ ID NO: 40 - protein, 8 aa, synthetic construct
  REGION 1..8: note = IgG Fc CH2 DE-TURN-4
EQYNSTFR

SEQ ID NO: 41 - protein, 109 aa, synthetic construct
  REGION 1..109: note = DB-B63 IgG Fc-CH2
DSNPRGVSVFLFPPKPKDTLMISRTPEVTCVVVDLAPSKGTVNFNWYVDGVEVHNAKTKPREKQRNGTLTVVSVLTVLHQDWLNGKEYKCRVTHPHLPRALEKTISKAK

SEQ ID NO: 42 - protein, 110 aa, synthetic construct
  REGION 1..110: note = DB-B64 IgG Fc-CH2
APELLGGPSVFLFPPKPKDTLMISRTPEVTCVVVDLAPSKGTVKFNWYVDGVEVHNAKTKPREKQRNGTLTVVSVLTVLHQDWLNGKEYKCKVTHPHLPRALEKTISKAK